European Patent Application EP 4 223 780 A1, published August 9, 2023. Title: ANTI-CD22 ANTIBODY MOLECULE OR ANTIGEN-BINDING FRAGMENT AND USE THEREOF. Applicant: KUNMING SINOWAY NATURAL PHARMACEUTICALS CO., LTD. The sequence listing filed with the application follows.

SEQUENCE LISTING (26 sequences)

SEQ ID NO: 1 - protein, 123 aa, artificial sequence
  HA22 VH
EVQLVESGGGLVKPGGSLKLSCAASGFAFSIYDMSWVRQTPEKCLEWVAYISSGGGTTYYPDTVKGRFTISRDNAKNTLYLQMSSLKSEDTAMYYCARHSGYGTHWGVLFAYWGQGTLVTVSA

SEQ ID NO: 2 - protein, 107 aa, artificial sequence
  HA22 VL
DIQMTQTTSSLSASLGDRVTISCRASQDISNYLNWYQQKPDGTVKLLIYYTSILHSGVPSRFSGSGSGTDYSLTISNLEQEDFATYFCQQGNTLPWTFGCGTKLEIK

SEQ ID NO: 3 - protein, 123 aa, artificial sequence
  VH1
EVQLVESGGGLVKPGGSLRLSCAASGFAFSIYDMSWVRQAPGKCLEWVAYISSGGGTTYYPDSVKGRFTISRENAKNSLYLQMNSLKSEDTAMYYCARHSGYGTHWGVLFAYWGQGTMVTVSS

SEQ ID NO: 4 - protein, 123 aa, artificial sequence
  VH2
EVQLVESGGGLVKPGGSLRLSCAASGFAFSIYDMSWVRQTPEKCLEWVAYISSGGGTTYYPDSVKGRFTISRENAKNSLYLQMNSLKSEDTAMYYCARHSGYGTHWGVLFAYWGQGTMVTVSS

SEQ ID NO: 5 - protein, 123 aa, artificial sequence
  VH4
EVQLVESGGGLVKPGGSLRLSCAASGFAFSIYDMSWIRQAPGKCLEWVAYISSGGGTTYYPGSVKGRFTISRENAKNSLYLQMNSLRAGDTAVYYCARHSGYGTHWGVLFAYWGQGTMVTVSS

SEQ ID NO: 6 - protein, 123 aa, artificial sequence
  VH5
EVQLVESGGGLVKPGGSLRLSCAASGFAFSIYDMSWIRQAPGKCLEWVAYISSGGGTTYYPGSVKGRFTISRENAKNSLYLQMNSLRSEDTAVYYCARHSGYGTHWGVLFAYWGQGTMVTVSS

SEQ ID NO: 7 - protein, 107 aa, artificial sequence
  VL-2
DIQMTQSTSTLSASVGDRVTITCRASQDISNYLNWYQQRPDGSVKLLIYYTSILHSGVPSRFSGSGSGTDYTLTISSLQDEDFATYFCQQGNTLPWTFGCGTKVEIK

SEQ ID NO: 8 - protein, 107 aa, artificial sequence
  VL-4
DIQMTQSPSTLSASVGDRVTITCRASQDISNYLNWFQQRPGQSPRLLIYYTSILHSGVPSRFSGSGSGTDYTLTISSLQPEDFATYYCQQGNTLPWTFGCGTKVEIK

SEQ ID NO: 9 - protein, 107 aa, artificial sequence [sequence omitted]

SEQ ID NO: 10 - protein, 330 aa, artificial sequence [sequence omitted]

SEQ ID NO: 11 - protein, 453 aa, artificial sequence
  HA22 HC
EVQLVESGGGLVKPGGSLKLSCAASGFAFSIYDMSWVRQTPEKCLEWVAYISSGGGTTYYPDTVKGRFTISRDNAKNTLYLQMSSLKSEDTAMYYCARHSGYGTHWGVLFAYWGQGTLVTVSAASTKGPSVFPLAPSSKSTSGGTAALGCLVKDYFPEPVTVSWNSGALTSGVHTFPAVLQSSGLYSLSSVVTVPSSSLGTQTYICNVNHKPSNTKVDKKVEPKSCDKTHTCPPCPAPELLGGPSVFLFPPKPKDTLMISRTPEVTCVVVDVSHEDPEVKFNWYVDGVEVHNAKTKPREEQYNSTYRVVSVLTVLHQDWLNGKEYKCKVSNKALPAPIEKTISKAKGQPREPQVYTLPPSRDELTKNQVSLTCLVKGFYPSDIAVEWESNGQPENNYKTTPPVLDSDGSFFLYSKLTVDKSRWQQGNVFSCSVMHEALHNHYTQKSLSLSPGK

SEQ ID NO: 12 - protein, 214 aa, artificial sequence
  HA22 LC
DIQMTQTTSSLSASLGDRVTISCRASQDISNYLNWYQQKPDGTVKLLIYYTSILHSGVPSRFSGSGSGTDYSLTISNLEQEDFATYFCQQGNTLPWTFGCGTKLEIKRTVAAPSVFIFPPSDEQLKSGTASVVCLLNNFYPREAKVQWKVDNALQSGNSQESVTEQDSKDSTYSLSSTLTLSKADYEKHKVYACEVTHQGLSSPVTKSFNRGEC

SEQ ID NO: 13 - protein, 453 aa, artificial sequence
  V2 HC
EVQLVESGGGLVKPGGSLRLSCAASGFAFSIYDMSWVRQTPEKCLEWVAYISSGGGTTYYPDSVKGRFTISRENAKNSLYLQMNSLKSEDTAMYYCARHSGYGTHWGVLFAYWGQGTMVTVSSASTKGPSVFPLAPSSKSTSGGTAALGCLVKDYFPEPVTVSWNSGALTSGVHTFPAVLQSSGLYSLSSVVTVPSSSLGTQTYICNVNHKPSNTKVDKKVEPKSCDKTHTCPPCPAPELLGGPSVFLFPPKPKDTLMISRTPEVTCVVVDVSHEDPEVKFNWYVDGVEVHNAKTKPREEQYNSTYRVVSVLTVLHQDWLNGKEYKCKVSNKALPAPIEKTISKAKGQPREPQVYTLPPSRDELTKNQVSLTCLVKGFYPSDIAVEWESNGQPENNYKTTPPVLDSDGSFFLYSKLTVDKSRWQQGNVFSCSVMHEALHNHYTQKSLSLSPGK

SEQ ID NO: 14 - protein, 214 aa, artificial sequence
  V2 LC
DIQMTQSTSTLSASVGDRVTITCRASQDISNYLNWYQQRPDGSVKLLIYYTSILHSGVPSRFSGSGSGTDYTLTISSLQDEDFATYFCQQGNTLPWTFGCGTKVEIKRTVAAPSVFIFPPSDEQLKSGTASVVCLLNNFYPREAKVQWKVDNALQSGNSQESVTEQDSKDSTYSLSSTLTLSKADYEKHKVYACEVTHQGLSSPVTKSFNRGEC

SEQ ID NO: 15 - protein, 453 aa, artificial sequence
  V1 HC
EVQLVESGGGLVKPGGSLRLSCAASGFAFSIYDMSWVRQAPGKCLEWVAYISSGGGTTYYPDSVKGRFTISRENAKNSLYLQMNSLKSEDTAMYYCARHSGYGTHWGVLFAYWGQGTMVTVSSASTKGPSVFPLAPSSKSTSGGTAALGCLVKDYFPEPVTVSWNSGALTSGVHTFPAVLQSSGLYSLSSVVTVPSSSLGTQTYICNVNHKPSNTKVDKKVEPKSCDKTHTCPPCPAPELLGGPSVFLFPPKPKDTLMISRTPEVTCVVVDVSHEDPEVKFNWYVDGVEVHNAKTKPREEQYNSTYRVVSVLTVLHQDWLNGKEYKCKVSNKALPAPIEKTISKAKGQPREPQVYTLPPSRDELTKNQVSLTCLVKGFYPSDIAVEWESNGQPENNYKTTPPVLDSDGSFFLYSKLTVDKSRWQQGNVFSCSVMHEALHNHYTQKSLSLSPGK

SEQ ID NO: 16 - protein, 214 aa, artificial sequence
  V4 LC
DIQMTQSPSTLSASVGDRVTITCRASQDISNYLNWFQQRPGQSPRLLIYYTSILHSGVPSRFSGSGSGTDYTLTISSLQPEDFATYYCQQGNTLPWTFGCGTKVEIKRTVAAPSVFIFPPSDEQLKSGTASVVCLLNNFYPREAKVQWKVDNALQSGNSQESVTEQDSKDSTYSLSSTLTLSKADYEKHKVYACEVTHQGLSSPVTKSFNRGEC

SEQ ID NO: 17 - protein, 453 aa, artificial sequence
  V5 HC
EVQLVESGGGLVKPGGSLRLSCAASGFAFSIYDMSWIRQAPGKCLEWVAYISSGGGTTYYPGSVKGRFTISRENAKNSLYLQMNSLRSEDTAVYYCARHSGYGTHWGVLFAYWGQGTMVTVSSASTKGPSVFPLAPSSKSTSGGTAALGCLVKDYFPEPVTVSWNSGALTSGVHTFPAVLQSSGLYSLSSVVTVPSSSLGTQTYICNVNHKPSNTKVDKKVEPKSCDKTHTCPPCPAPELLGGPSVFLFPPKPKDTLMISRTPEVTCVVVDVSHEDPEVKFNWYVDGVEVHNAKTKPREEQYNSTYRVVSVLTVLHQDWLNGKEYKCKVSNKALPAPIEKTISKAKGQPREPQVYTLPPSRDELTKNQVSLTCLVKGFYPSDIAVEWESNGQPENNYKTTPPVLDSDGSFFLYSKLTVDKSRWQQGNVFSCSVMHEALHNHYTQKSLSLSPGK

SEQ ID NO: 18 - protein, 453 aa, artificial sequence
  V4 HC
EVQLVESGGGLVKPGGSLRLSCAASGFAFSIYDMSWIRQAPGKCLEWVAYISSGGGTTYYPGSVKGRFTISRENAKNSLYLQMNSLRAGDTAVYYCARHSGYGTHWGVLFAYWGQGTMVTVSSASTKGPSVFPLAPSSKSTSGGTAALGCLVKDYFPEPVTVSWNSGALTSGVHTFPAVLQSSGLYSLSSVVTVPSSSLGTQTYICNVNHKPSNTKVDKKVEPKSCDKTHTCPPCPAPELLGGPSVFLFPPKPKDTLMISRTPEVTCVVVDVSHEDPEVKFNWYVDGVEVHNAKTKPREEQYNSTYRVVSVLTVLHQDWLNGKEYKCKVSNKALPAPIEKTISKAKGQPREPQVYTLPPSRDELTKNQVSLTCLVKGFYPSDIAVEWESNGQPENNYKTTPPVLDSDGSFFLYSKLTVDKSRWQQGNVFSCSVMHEALHNHYTQKSLSLSPGK

SEQ ID NO: 19 - protein, 5 aa, artificial sequence
  H-CDR1
IYDMS

SEQ ID NO: 20 - protein, 17 aa, artificial sequence
  H-CDR2
YISSGGGTTYYPDTVKG

SEQ ID NO: 21 - protein, 14 aa, artificial sequence
  H-CDR3
HSGYGTHWGVLFAY

SEQ ID NO: 22 - protein, 11 aa, artificial sequence
  L-CDR1
RASQDISNYLN

SEQ ID NO: 23 - protein, 7 aa, artificial sequence
  L-CDR2
YTSILHS

SEQ ID NO: 24 - protein, 9 aa, artificial sequence
  L-CDR3
QQGNTLPWT

SEQ ID NO: 25 - protein, 17 aa, artificial sequence
  H-CDR2
YISSGGGTTYYPDSVKG

SEQ ID NO: 26 - protein, 17 aa, artificial sequence
  H-CDR2
YISSGGGTTYYPGSVKG